European Patent Application EP 4 759 331 A2, published June 17, 2026. Title: MeCP2 expression cassettes. Applicant: The University Court of the University of Glasgow. The sequence listing filed with the application follows.

SEQUENCE LISTING (32 sequences)

SEQ ID NO: 1 - DNA, 104 bp, synthetic construct
  misc_feature 1..104: note = scAAV vector containing AAV-2 ITR
  source 1..104: mol_type = other DNA
gcgcgctcgctcgctcactgaggccgcccgggcaaagcccgggcgtcgggcgacctttggtcgcccggcctcagtgagcgagcgagcgcgcagagagggagtgg

SEQ ID NO: 2 - DNA, 104 bp, synthetic construct
  misc_feature 1..104: note = scAAV vector containing AVV-2 ITRs
  source 1..104: mol_type = other DNA
ccactccctctctgcgcgctcgctcgctcactgaggccgggcgaccaaaggtcgcccgacgcccgggctttgcccgggcggcctcagtgagcgagcgagcgcgc

SEQ ID NO: 3 - protein, 499 aa, synthetic construct
  REGION 1..499: note = Human MeCP2 protein isoform 1
MAAAAAAAPSGGGGGGEEERLEEKSEDQDLQGLKDKPLKFKKVKKDKKEEKEGKHEPVQPSAHHSAEPAEAGKAETSEGSGSAPAVPEASASPKQRRSIIRDRGPMYDDPTLPEGWTRKLKQRKSGRSAGKYDVYLINPQGKAFRSKVELIAYFEKVGDTSLDPNDFDFTVTGRGSPSRREQKPPKKPKSPKAPGTGRGRGRPKGSGTTRPKAATSEGVQVKRVLEKSPGKLLVKMPFQTSPGGKAEGGGATTSTQVMVIKRPGRKRKAEADPQAIPKKRGRKPGSVVAAAAAEAKKKAVKESSIRSVQETVLPIKKRKTRETVSIEVKEVVKPLLVSTLGEKSGKGLKTCKSPGRKSKESSPKGRSSSASSPPKKEHHHHHHHSESPKAPVPLLPPLPPPPPEPESSEDPTSPPEPQDLSSSVCKEEKMPRGGSLESDGCPKEPAKTQPAVATAATAAEKYKHRGEGERKDIVSSSMPRPNREEPVDSRTPVTERVSS

SEQ ID NO: 4 - protein, 487 aa, synthetic construct
  REGION 1..487: note = Human MeCP2 protein isoform 2
MVAGMLGLREEKSEDQDLQGLKDKPLKFKKVKKDKKEEKEGKHEPVQPSAHHSAEPAEAGKAETSEGSGSAPAVPEASASPKQRRSIIRDRGPMYDDPTLPEGWTRKLKQRKSGRSAGKYDVYLINPQGKAFRSKVELIAYFEKVGDTSLDPNDFDFTVTGRGSPSRREQKPPKKPKSPKAPGTGRGRGRPKGSGTTRPKAATSEGVQVKRVLEKSPGKLLVKMPFQTSPGGKAEGGGATTSTQVMVIKRPGRKRKAEADPQAIPKKRGRKPGSVVAAAAAEAKKKAVKESSIRSVQETVLPIKKRKTRETVSIEVKEVVKPLLVSTLGEKSGKGLKTCKSPGRKSKESSPKGRSSSASSPPKKEHHHHHHHSESPKAPVPLLPPLPPPPPEPESSEDPTSPPEPQDLSSSVCKEEKMPRGGSLESDGCPKEPAKTQPAVATAATAAEKYKHRGEGERKDIVSSSMPRPNREEPVDSRTPVTERVSS

SEQ ID NO: 5 - protein, 102 aa, synthetic construct
  REGION 1..102: note = methyl-CpG binding domain (MBD) of human MeCP protein
PAVPEASASPKQRRSIIRDRGPMYDDPTLPEGWTRKLKQRKSGRSAGKYDVYLINPQGKAFRSKVELIAYFEKVGDTSLDPNDFDFTVTGRGSPSRREQKPP

SEQ ID NO: 6 - protein, 40 aa, synthetic construct
  REGION 1..40: note = NCoR/SMRT Interaction Domain (NID) of human MeCP2
PGSVVAAAAAEAKKAVKESSIRSVQETVLPIKKRKTRETV

SEQ ID NO: 7 - protein, 17 aa, synthetic construct
  REGION 1..17: note = native MeCP2 NLS
RKAEADPQAIPKKRGRK

SEQ ID NO: 8 - protein, 7 aa, synthetic construct
  REGION 1..7: note = SV40 Large T antigen NLS
PKKKRKV

SEQ ID NO: 9 - protein, 475 aa, synthetic construct
  REGION 1..475: note = MeCP2
SEDQDLQGLKDKPLKFKKVKKDKKEEKEGKHEPVQPSAHHSAEPAEAGKAETSEGSGSAPAVPEASASPKQRRSIIRDRGPMYDDPTLPEGWTRKLKQRKSGRSAGKYDVYLINPQGKAFRSKVELIAYFEKVGDTSLDPNDFDFTVTGRGSPSRREQKPPKKPKSPKAPGTGRGRGRPKGSGTTRPKAATSEGVQVKRVLEKSPGKLLVKMPFQTSPGGKAEGGGATTSTQVMVIKRPGRKRKAEADPQAIPKKRGRKPGSVVAAAAAEAKKKAVKESSIRSVQETVLPIKKRKTRETVSIEVKEVVKPLLVSTLGEKSGKGLKTCKSPGRKSKESSPKGRSSSASSPPKKEHHHHHHHSESPKAPVPLLPPLPPPPPEPESSEDPTSPPEPQDLSSSVCKEEKMPRGGSLESDGCPKEPAKTQPAVATAATAAEKYKHRGEGERKDIVSSSMPRPNREEPVDSRTPVTERVSS

SEQ ID NO: 10 - protein, 241 aa, synthetic construct
  REGION 1..241: note = MeCP2 fragment designated Delta NC
PAVPEASASPKQRRSIIRDRGPMYDDPTLPEGWTRKLKQRKSGRSAGKYDVYLINPQGKAFRSKVELIAYFEKVGDTSLDPNDFDFTVTGRGSPSRREQKPPKKPKSPKAPGTGRGRGRPKGSGTTRPKAATSEGVQVKRVLEKSPGKLLVKMPFQTSPGGKAEGGGATTSTQVMVIKRPGRKRKAEADPQAIPKKRGRKPGSVVAAAAAEAKKKAVKESSIRSVQETVLPIKKRKTRETV

SEQ ID NO: 11 - protein, 157 aa, synthetic construct
  REGION 1..157: note = Protein variant designated Delta NIC
PAVPEASASPKQRRSIIRDRGPMYDDPTLPEGWTRKLKQRKSGRSAGKYDVYLINPQGKAFRSKVELIAYFEKVGDTSLDPNDFDFTVTGRGSPSRREQKPPGSSGSSGPKKKRKVPGSVVAAAAAEAKKKAVKESSIRSVQETVLPIKKRKTRETV

SEQ ID NO: 12 - protein, 24 aa, synthetic construct
  REGION 1..24: note = N-terminal portion
MAAAAAAAPSGGGGGGEEERLEEK

SEQ ID NO: 13 - protein, 12 aa, synthetic construct
  REGION 1..12: note = N-terminal portion
MVAGMLGLREEK

SEQ ID NO: 14 - protein, 499 aa, synthetic construct; identical to SEQ ID NO: 3
  REGION 1..499: note = MeCP2 protein encoded by the expression cassette, human isoform 1

SEQ ID NO: 15 - protein, 487 aa, synthetic construct; identical to SEQ ID NO: 4
  REGION 1..487: note = MeCP2 protein encoded by the expression cassette, human isoform 2

SEQ ID NO: 16 - protein, 265 aa, synthetic construct
  REGION 1..265: note = MeCP2 protein encoded by the expression cassette Delta NC isoform 1
MAAAAAAAPSGGGGGGEEERLEEKPAVPEASASPKQRRSIIRDRGPMYDDPTLPEGWTRKLKQRKSGRSAGKYDVYLINPQGKAFRSKVELIAYFEKVGDTSLDPNDFDFTVTGRGSPSRREQKPPKKPKSPKAPGTGRGRGRPKGSGTTRPKAATSEGVQVKRVLEKSPGKLLVKMPFQTSPGGKAEGGGATTSTQVMVIKRPGRKRKAEADPQAIPKKRGRKPGSVVAAAAAEAKKKAVKESSIRSVQETVLPIKKRKTRETV

SEQ ID NO: 17 - protein, 253 aa, synthetic construct
  REGION 1..253: note = MeCP2 protein encoded by the expression cassette Delta NC isoform 2
MVAGMLGLREEKPAVPEASASPKQRRSIIRDRGPMYDDPTLPEGWTRKLKQRKSGRSAGKYDVYLINPQGKAFRSKVELIAYFEKVGDTSLDPNDFDFTVTGRGSPSRREQKPPKKPKSPKAPGTGRGRGRPKGSGTTRPKAATSEGVQVKRVLEKSPGKLLVKMPFQTSPGGKAEGGGATTSTQVMVIKRPGRKRKAEADPQAIPKKRGRKPGSVVAAAAAEAKKKAVKESSIRSVQETVLPIKKRKTRETV

SEQ ID NO: 18 - protein, 181 aa, synthetic construct
  REGION 1..181: note = MeCP2 protein encoded by the expression cassette, Delta NIC isoform 1
MAAAAAAAPSGGGGGGEEERLEEKPAVPEASASPKQRRSIIRDRGPMYDDPTLPEGWTRKLKQRKSGRSAGKYDVYLINPQGKAFRSKVELIAYFEKVGDTSLDPNDFDFTVTGRGSPSRREQKPPGSSGSSGPKKKRKVPGSVVAAAAAEAKKKAVKESSIRSVQETVLPIKKRKTRETV

SEQ ID NO: 19 - protein, 169 aa, synthetic construct
  REGION 1..169: note = MeCP2 protein encoded by the expression cassette, Delta NIC isoform 2
MVAGMLGLREEKPAVPEASASPKQRRSIIRDRGPMYDDPTLPEGWTRKLKQRKSGRSAGKYDVYLINPQGKAFRSKVELIAYFEKVGDTSLDPNDFDFTVTGRGSPSRREQKPPGSSGSSGPKKKRKVPGSVVAAAAAEAKKKAVKESSIRSVQETVLPIKKRKTRETV

SEQ ID NO: 20 - protein, 10 aa, synthetic construct
  REGION 1..10: note = C-terminal c-Myc epitope tag
EQKLISEEDL

SEQ ID NO: 21 - protein, 515 aa, synthetic construct
  REGION 1..515: note = MeCP2 protein comprising a heterologous sequence
MAAAAAAAPSGGGGGGEEERLEEKSEDQDLQGLKDKPLKFKKVKKDKKEEKEGKHEPVQPSAHHSAEPAEAGKAETSEGSGSAPAVPEASASPKQRRSIIRDRGPMYDDPTLPEGWTRKLKQRKSGRSAGKYDVYLINPQGKAFRSKVELIAYFEKVGDTSLDPNDFDFTVTGRGSPSRREQKPPKKPKSPKAPGTGRGRGRPKGSGTTRPKAATSEGVQVKRVLEKSPGKLLVKMPFQTSPGGKAEGGGATTSTQVMVIKRPGRKRKAEADPQAIPKKRGRKPGSVVAAAAAEAKKKAVKESSIRSVQETVLPIKKRKTRETVSIEVKEVVKPLLVSTLGEKSGKGLKTCKSPGRKSKESSPKGRSSSASSPPKKEHHHHHHHSESPKAPVPLLPPLPPPPPEPESSEDPTSPPEPQDLSSSVCKEEKMPRGGSLESDGCPKEPAKTQPAVATAATAAEKYKHRGEGERKDIVSSSMPRPNREEPVDSRTPVTERVSSRGPFEQKLISEEDLVD

SEQ ID NO: 22 - protein, 284 aa, synthetic construct
  REGION 1..284: note = A c-Myc-tagged version of the Delta NC protein
MAAAAAAAPSGGGGGGEEERLEEKPAVPEASASPKQRRSIIRDRGPMYDDPTLPEGWTRKLKQRKSGRSAGKYDVYLINPQGKAFRSKVELIAYFEKVGDTSLDPNDFDFTVTGRGSPSRREQKPPKKPKSPKAPGTGRGRGRPKGSGTTRPKAATSEGVQVKRVLEKSPGKLLVKMPFQTSPGGKAEGGGATTSTQVMVIKRPGRKRKAEADPQAIPKKRGRKPGSVVAAAAAEAKKKAVKESSIRSVQETVLPIKKRKTRETVGSSGSSGEQKLISEEDLVD

SEQ ID NO: 23 - protein, 200 aa, synthetic construct
  REGION 1..200: note = c-Myc-tagged version of the Delta NIC protein
MAAAAAAAPSGGGGGGEEERLEEKPAVPEASASPKQRRSIIRDRGPMYDDPTLPEGWTRKLKQRKSGRSAGKYDVYLINPQGKAFRSKVELIAYFEKVGDTSLDPNDFDFTVTGRGSPSRREQKPPGSSGSSGPKKKRKVPGSVVAAAAAEAKKKAVKESSIRSVQETVLPIKKRKTRETVGSSGSSGEQKLISEEDLVD

SEQ ID NO: 24 - protein, 130 aa, synthetic construct
  REGION 1..130: note = 5' transcriptional control comprising a core promoter element
AAACCAGCCCCTCTGTGCCCTAGCCGCCTCTTTTTTCCAAGTGACAGTAGAACTCCACCAATCCGCAGCTGAATGGGGTCCGCCTCTTTTCCCTGCCTAAACAGACAGGAACTCCTGCCAATTGAGGGCG

SEQ ID NO: 25 - DNA, 62 bp, synthetic construct
  misc_feature 1..62: note = 5' transcriptional control region comprising a silencer element
  source 1..62: mol_type = other DNA
ttaagcgccagagtccacaagggcccagttaatcctcaacattcaaatgctgcccacaaaac

SEQ ID NO: 26 - DNA, 19 bp, synthetic construct
  misc_feature 1..19: note = 5' transcriptional control region comprising a CNS regulatory element
  source 1..19: mol_type = other DNA
cagcacacaggctggtcgg

SEQ ID NO: 27 - DNA, 29 bp, synthetic construct
  misc_feature 1..29: note = a miR-22 binding site
  source 1..29: mol_type = other DNA
acaagaataaaggcagctgttgtctcttc

SEQ ID NO: 28 - DNA, 30 bp, synthetic construct
  misc_feature 1..30: note = a miR-19 binding site
  source 1..30: mol_type = other DNA
agaagtagctttgcacttttctaaactagg

SEQ ID NO: 29 - DNA, 30 bp, synthetic construct
  misc_feature 1..30: note = a miR-132 binding site
  source 1..30: mol_type = other DNA
aatatcaccaggactgttactcaatgtgtg

SEQ ID NO: 30 - RNA, 13 nt, synthetic construct
  misc_feature 1..13: note = 3'UTR of the MeCP2 gene, AU-rich element
  source 1..13: mol_type = other RNA
atatatttaaaaa

SEQ ID NO: 31 - RNA, 23 nt, synthetic construct
  misc_feature 1..23: note = MeCP2 gene, GU-rich region
  source 1..23: mol_type = other RNA
tgtccgtttgtgtcttttgttgt

SEQ ID NO: 32 - DNA, 6043 bp, synthetic construct
  misc_feature 1..6043: note = 2nd generation expression cassette
  source 1..6043: mol_type = other DNA
tgcgcgctcgctcgctcactgaggccgcccgggcaaagcccgggcgtcgggcgacctttggtcgcccggcctcagtgagcgagcgagcgcgcagagagggagtggggttcggtacccataggcgccaagagcctagacttccttaagcgccagagtccacaagggcccagttaatcctcaacattcaaatgctgcccacaaaaccagcccctctgtgccctagccgcctcttttttccaagtgacagtagaactccaccaatccgcagctgaatggggtccgcctcttttccctgcctaaacagacaggaactcctgccaattgagggcgtcaccgctaaggctccgccccagcctgggctccacaaccaatgaagggtaatctcgacaaagagcaaggggtggggcgcgggcgcgcaggtgcagcagcacacaggctggtcgggagggcggggcgcgacgtctgccgtgcggggtcccggcatcggttgcgcgcgcgctccctcctctcggagagagggctgtggtaaaacccgtccggaaaccatggccgccgccgccgccgccgcgccgagcggaggaggaggaggaggcgaggaggagagactggaagaaaagtcagaagaccaggacctccagggcctcaaggacaaacccctcaagtttaaaaaggtgaagaaagataagaaagaagagaaagagggcaagcatgagcccgtgcagccatcagcccaccactctgctgagcccgcagaggcaggcaaagcagagacatcagaagggtcaggctccgccccggctgtgccggaagcttctgcctcccccaaacagcggcgctccatcatccgtgaccggggacccatgtatgatgaccccaccctgcctgaaggctggacacggaagcttaagcaaaggaaatctggccgctctgctgggaagtatgatgtgtatttgatcaatccccagggaaaagcctttcgctctaaagtggagttgattgcgtacttcgaaaaggtaggcgacacatccctggaccctaatgattttgacttcacggtaactgggagagggagcccctcccggcgagagcagaaaccacctaagaagcccaaatctcccaaagctccaggaactggcagaggccggggacgccccaaagggagcggcaccacgagacccaaggcggccacgtcagagggtgtgcaggtgaaaagggtcctggagaaaagtcctgggaagctccttgtcaagatgccttttcaaacttcgccagggggcaaggctgaggggggtggggccaccacatccacccaggtcatggtgatcaaacgccccggcaggaagcgaaaagctgaggccgaccctcaggccattcccaagaaacggggccgaaagccggggagtgtggtggcagccgctgccgccgaggccaaaaagaaagccgtgaaggagtcttctatccgatctgtgcaggagaccgtactccccatcaagaagcgcaagacccgggagacggtcagcatcgaggtcaaggaagtggtgaagcccctgctggtgtccaccctcggtgagaagagcgggaaaggactgaagacctgtaagagccctgggcggaaaagcaaggagagcagccccaaggggcgcagcagcagcgcctcctcaccccccaagaaggagcaccaccaccatcaccaccactcagagtccccaaaggcccccgtgccactgctcccacccctgcccccacctccacctgagcccgagagctccgaggaccccaccagcccccctgagccccaggacttgagcagcagcgtctgcaaagaggagaagatgcccagaggaggctcactggagagcgacggctgccccaaggagccagctaagactcagcccgcggttgccaccgccgccacggccgcagaaaagtacaaacaccgaggggagggagagcgcaaagacattgtttcatcctccatgccaaggccaaacagagaggagcctgtggacagccggacgcccgtgaccgagagagttagctctagagggcccttcgaacaaaaactcatctcagaagaggatctggtcgactagagctcgctgatcagcctcacaagaataaaggcagctgttgtctcttcagaagtagctttgcacttttctaaactaggaatatcaccaggactgttactcaatgtgtgggtaccgaaagcactgatatatttaaaaacaaaaggtgtaacctatttattatataaagagtttgccttataaatttacataaaaatgtccgtttgtgtcttttgttgtaaaaatcacgcgtaggaacccctagtgatggagttggccactccctctctgcgcgctcgctcgctcactgaggccgggcgaccaaaggtcgcccgacgcccgggctttgcccgggcggcctcagtgagcgagcgagcgcgcagctggcgtaatagcgaagaggcccgcaccgatcgcccttcccaacagttgcgcagcctgaatggcgaatggcgattccgttgcaatggctggcggtaatattgttctggatattaccagcaaggccgatagtttgagttcttctactcaggcaagtgatgttattactaatcaaagaagtattgcgacaacggttaatttgcgtgatggacagactcttttactcggtggcctcactgattataaaaacacttctcaggattctggcgtaccgttcctgtctaaaatccctttaatcggcctcctgtttagctcccgctctgattctaacgaggaaagcacgttatacgtgctcgtcaaagcaaccatagtacgcgccctgtagcggcgcattaagcgcggcgggtgtggtggttacgcgcagcgtgaccgctacacttgccagcgccctagcgcccgctcctttcgctttcttcccttcctttctcgccacgttcgccggctttccccgtcaagctctaaatcgggggctccctttagggttccgatttagtgctttacggcacctcgaccccaaaaaacttgattagggtgatggttcacgtagtgggccatcgccctgatagacggtttttcgccctttgacgttggagtccacgttctttaatagtggactcttgttccaaactggaacaacactcaaccctatctcggtctattcttttgatttataagggattttgccgatttcggcctattggttaaaaaatgagctgatttaacaaaaatttaacgcgaattttaacaaaatattaacgcttacaatttaaatatttgcttatacaatcttcctgtttttggggcttttctgattatcaaccggggtacatatgattgacatgctagttttacgattaccgttcatcgattctcttgtttgctccagactctcaggcaatgacctgatagcctttgtagagacctctcaaaaatagctaccctctccggcatgaatttatcagctagaacggttgaatatcatattgatggtgatttgactgtctccggcctttctcacccgtttgaatctttacctacacattactcaggcattgcatttaaaatatatgagggttctaaaaatttttatccttgcgttgaaataaaggcttctcccgcaaaagtattacagggtcataatgtttttggtacaaccgatttagctttatgctctgaggctttattgcttaattttgctaattctttgccttgcctgtatgatttattggatgttggaattcctgatgcggtattttctccttacgcatctgtgcggtatttcacaccgcatatggtgcactctcagtacaatctgctctgatgccgcatagttaagccagccccgacacccgccaacacccgctgacgcgccctgacgggcttgtctgctcccggcatccgcttacagacaagctgtgaccgtctccgggagctgcatgtgtcagaggttttcaccgtcatcaccgaaacgcgcgagacgaaagggcctcgtgatacgcctatttttataggttaatgtcatgataataatggtttcttagacgtcaggtggcacttttcggggaaatgtgcgcggaacccctatttgtttatttttctaaatacattcaaatatgtatccgctcatgagacaataaccctgataaatgcttcaataatattgaaaaaggaagagtatgagtattcaacatttccgtgtcgcccttattcccttttttgcggcattttgccttcctgtttttgctcacccagaaacgctggtgaaagtaaaagatgctgaagatcagttgggtgcacgagtgggttacatcgaactggatctcaacagcggtaagatccttgagagttttcgccccgaagaacgttttccaatgatgagcacttttaaagttctgctatgtggcgcggtattatcccgtattgacgccgggcaagagcaactcggtcgccgcatacactattctcagaatgacttggttgagtactcaccagtcacagaaaagcatcttacggatggcatgacagtaagagaattatgcagtgctgccataaccatgagtgataacactgcggccaacttacttctgacaacgatcggaggaccgaaggagctaaccgcttttttgcacaacatgggggatcatgtaactcgccttgatcgttgggaaccggagctgaatgaagccataccaaacgacgagcgtgacaccacgatgcctgtagcaatggcaacaacgttgcgcaaactattaactggcgaactacttactctagcttcccggcaacaattaatagactggatggaggcggataaagttgcaggaccacttctgcgctcggcccttccggctggctggtttattgctgataaatctggagccggtgagcgtgggtctcgcggtatcattgcagcactggggccagatggtaagccctcccgtatcgtagttatctacacgacggggagtcaggcaactatggatgaacgaaatagacagatcgctgagataggtgcctcactgattaagcattggtaactgtcagaccaagtttactcatatatactttagattgatttaaaacttcatttttaatttaaaaggatctaggtgaagatcctttttgataatctcatgaccaaaatcccttaacgtgagttttcgttccactgagcgtcagaccccgtagaaaagatcaaaggatcttcttgagatcctttttttctgcgcgtaatctgctgcttgcaaacaaaaaaaccaccgctaccagcggtggtttgtttgccggatcaagagctaccaactctttttccgaaggtaactggcttcagcagagcgcagataccaaatactgtccttctagtgtagccgtagttaggccaccacttcaagaactctgtagcaccgcctacatacctcgctctgctaatcctgttaccagtggctgctgccagtggcgataagtcgtgtcttaccgggttggactcaagacgatagttaccggataaggcgcagcggtcgggctgaacggggggttcgtgcacacagcccagcttggagcgaacgacctacaccgaactgagatacctacagcgtgagctatgagaaagcgccacgcttcccgaagggagaaaggcggacaggtatccggtaagcggcagggtcggaacaggagagcgcacgagggagcttccagggggaaacgcctggtatctttatagtcctgtcgggtttcgccacctctgacttgagcgtcgatttttgtgatgctcgtcaggggggcggagcctatggaaaaacgccagcaacgcggcctttttacggttcctggccttttgctggccttttgctcacatgttctttcctgcgttatcccctgattctgtggataaccgtattaccgcctttgagtgagctgataccgctcgccgcagccgaacgaccgagcgcagcgagtcagtgagcgaggaagcggaagagcgcccaatacgcaaaccgcctctccccgcgcgttggccgattcattaatgcagc